European Patent Application EP 4 265 729 A1, published October 25, 2023. Title: Microorganism with high productivity of tripeptide and use thereof. Applicant: SAMYANG COPORATION. The sequence listing filed with the application follows.

SEQUENCE LISTING (3 sequences)

SEQ ID NO: 1 - DNA, 473 bp, Artificial Sequence
  18S rDNA of Candida utilis
acctgggcctgcgcttctagcgcggctccaaccaatacacagtgtattttgcttcttttgctttggctctgccaaaggttttaaacacagaaatttattttctctagaaactagtcaatttgaattttaatcttcaaaactttcaacaacggatctcttggttctcgcaacgatgaagaacgcagcgaaatgcgatacgtaatgtgaattgcaggttttcgtgaatcatcgaatctttgaacgcatattgcgctctctggcattccagagagcatgcctgtttgagcgtcatttctctctcaagatcctctaggggacttggtattgagtgatactctgtgttaacttgaaatactctaggcagagctccccctagaaatcctctgggccgaaataatgtattaggttctaccaactcgttattttccagacagacttccaggcagagctcggctgaacaacctttctaagct

SEQ ID NO: 2 - DNA, 19 bp, Artificial Sequence
  Forward primer ITS1
tccgtaggtgaacctgcgg

SEQ ID NO: 3 - DNA, 19 bp, Artificial Sequence
  Backward primer ITS4
tccgtaggtgaacctgcgg